European Patent Application EP 4 378 600 A1, published June 5, 2024. Title: Method for biodegrading polyolefin-derived polymers. Applicant: Consejo Superior de Investigaciones Cientificas (CSIC). Application ES. The sequence listing filed with the application follows.

SEQUENCE LISTING (2 sequences)

SEQ ID NO: 1 - protein, 752 aa, Galleria mellonella
MVVTMRLVVAAVLLAAVAASVVHDELKNIVITKEPMKNMDMKSKEMCILKLMNHILQPTMYEDVREVAKAWVLEENEDKYMKMEAVKEFINTYKMGMLPRGEVFVHMDHKHVEEAVKVFKLLYFANDFDVFLKTACWLRERINGGMFVYALTAAIFHRSDCSGIKIPAPYEIYPYLFVDSNILHKAFMMKMSKAAMDPVMKNYYGIKVKDNSMVIIDWRKGLRHTMSEFDRTSYFTEDIDLNTYLYYMHMSYPYWMNEDMYRVNKERRGEAMWYGYQQLQARLRLERLSHHMCDLKPLDLDGTLDEGYWPKILLHTGDEMPVRYNKMKLTNENNIKYRLLLEDNKRLIRDGIKKGHMAMHDGTTVSLKKPDDIENLCRIVLGGFVSKDDHKGKSSIWRNLAKTMLSYGTYNMGKYTYIPTAADMYSTALRDPGMWKMLKLISEYFIMFKEMLPKYTREELDFPGVKIEQVTTDKLVTFMDEYDVDITNAVYLDHDEMQKHRSDMMYVARMHRLNHQPFKITIDVASDKAVECVVRVFLGPKLDCMGRFTSVNDKRNDMVEIDSFLYKLETGKNTIVRDSLEMNNVIKERPWSRNNWAMDPSGGQKAQDNWWYKSRIGFPHRLLLPMGSHGGMPYQMFVIVTPVRAGMSLPSIDMNTAKERKACRWTVCMDTMPLGFPFDRPIDETNFYTKNMKFHDVMVYTKDLAMSNMVKDVDMSEMVMKRDDLTYLDKDMLVKRSYKSVMMMSGDDMTHM

SEQ ID NO: 2 - protein, 702 aa, Galleria mellonella
MQTVLFLAALVSLAAAGYPQYHYDVETRKLDPSLLNIQTKVLSLLENWKQVNPDDEYYKIGKEYNVEANMESYTNREVVTEFLSLYKAGFIPKNEVFSIFYENQALEVIALYRLFYYAKDFETFYKTAAFARVWLNEGQFVYAFYLAVIHRADTRGIVLPAPYEIWPEYFMNSDVLSKIYRIQMQKGLIIPEQGPYYGILSKDNAYYFYANYSGPLTYEDNENLLSYFIEDIGWNSYYYYFHNRFPFWENGEQLIGPLKERRGEIYYYVYQKILARYYLERLANGLGEIPRFNWLDKYQTSYYPLLSSYQLPFAQRNDDYYLASGDNINDIQFIDTYEKTFLQLLQKGQFKAYKQEVDLYNSKSINFVGNYWQSNADLYEKVPKRNYWRSYEATARRVLGAAPRSSINYENMNIPTALDFYQTSLRDPAFYQLYAKILDYINEYKEYLEPYSQDVLHYVGVKINDVKVDKLVTYFEYFDWNATNAVYLSEQQLDTVSPSYIVRQPRLNNKPFTVNIDIKSDVESEVVVKIFLGPKYDGNGLPISLEDNWINFIELDWFTHKLTSGQNKIARKSEEFFFFKDDSVSLFKIYELLSNGQVPSYMVDRYIYLPRRLILPRGTQRGFPLQLFVVVYPYQAPVKEWESMRQYIVDNKPFGYPFDRPVTLPYYFNQPNMYFKDVYVYQEGEQYPYYNSYWSQNQVSNH